European Patent Application EP 4 116 418 A1, published January 11, 2023. Title: Compound and method for an allele-specific editing of the ELANE gene. Applicant: Eberhard Karls Universität - Medizinische Fakultät. The sequence listing filed with the application follows.

SEQUENCE LISTING (3 sequences)

SEQ ID NO: 1 - DNA, 20 bp, Artificial sequence
  V57 sgRNA
tcagggtgacgccgcagaag

SEQ ID NO: 2 - DNA, 20 bp, Artificial sequence
  V214 sgRNA
ggacgaaggaggcaattacg

SEQ ID NO: 3 - DNA, 183 bp, Artificial sequence
  ssODN repair template for ELANE G214V mutation
agagtcgatccagtttacaaactgtgccaccggggcaaaggcatcggggtagagccctgaggcgcagcctccccggacgaaggaggcaattccgtggattagcccgttgcagaccaaggggctgccggagtccccctgtggaggcagacaaggtggggaagctggactgcgaggccctgccca